European Patent Specification EP 4 065 708 B1, published January 3, 2024. Title: Method for digesting nucleic acid in a sample. Applicant: UEA Enterprises Limited. The sequence listing filed with the application follows.

SEQUENCE LISTING (2 sequences)

SEQ ID NO: 1 - protein, 213 aa, Artificial Sequence
  HL-SAN DNase
APPSSFSKAKKEAVKIYLDYPTEFYCGCDITWKNKKKGIPELESCGYQVRKQEKRASRIEWEHVVPAWQFGHQRQCWQKGGRKNCTRNDKQFKSMEADLHNLVPAIGEVNGDRSNFRFSQWNGSKGAFYGQCAFKVDFKGRVAEPPAQSRGAIARTYLYMNNEYKFNLSKAQRQLMEAWNKQYPVSTWECTRDERIAKIQGNHNQFVYKACTK

SEQ ID NO: 2 - protein, 209 aa, Artificial Sequence
  M-SAN DNase
APISFSHAKNEAVKIYRDHPVEFYCGCEIRWQGKKGIPDLESCGYQVRKNENRASRIEWEHVVPAWQFGHQLQCWQQGGRKNCTRTSPEFNQMEADLHNLVPAIGEVNGDRSNFRFSQWNSKGAFYGQCAFKVDFKGRVAEPPAQSRGAIARTYLYMSEQYGLRLSKAQNQLMQAWNNQYPVSEWECVRDQKIEKVQNSNRFVREQCPN